European Patent Application EP 4 692 314 A1, published February 11, 2026. Title: HOST CELL FOR IMPROVING STABILITY OF PLASMID. Applicant: Nanjing GenScript Biotech Co., Ltd. Application CN. The sequence listing filed with the application follows.

SEQUENCE LISTING (44 sequences)

SEQ ID NO: 1 - DNA, 3147 bp, Escherichia coli
  source 1..3147: mol_type = other DNA
ttatttcactgcaaacgtactttccagtttgctgtagcccaggccgttgatctttttcactttgatctgcaccggaatacgctctttcatcgcttctacgtggctaatcacaccgatggttttgccactggcgttcagggcatccagcgcatcaagggcggtatccagcgtttcgctatccagcgtgccaaaaccttcatcaaggaacagcgagtcaatacgtgttttatggctgaccagatccgaaagcgccagcgccagcgccagactaacgaggaaactttcgccgccggaaagggtacgggtatcgcgtaccgcatctgcctgccaggtatcaacaacctcgacttccagcgcctcgctggctttgcgctgtaacagatagcgcccgtgcagccgggtaagttgctgattagcgagatggactaaattatccagcgtcagcccctgggcaaacttgcggaatttatcgccctctttggaacctattagcgaattcagatatccccagtcctcaacctgctgcgtcatttgagcaatttgctgcattaaggtttgttgttgctgacggttatctgcatcctgcttcagctgctggcgaatctcgccttgactcgtggtgttttcacgcaacttttggtgagtttgcgctaactcttgctgaatctgctccaccgtcacagtgagagccaacccgtcgtcaggtcggtgttgttgatgctgtgccagcgtttctgctgtctgagtgaccagagtttgcgcctgacggcgctggttttccagattctgcttgagctgttccagctgcgttagtgtttgttcatccattagcgccgcaaggaacgcctgctgatcgtcaaagacgctggcctgtagcgcggtgtcaaactgcgcctgggctttttgcagactttgcgccgccagaacatcctgttgctgtaacgtctgctgctggctgtgtaatgcgagacattgttcatgtacctgccgccagttttccaataccacagtttcttcgcagtgcgggagttcatcactttgcggcaacgtttccagaatcggcgtcagctgctgaatacggttttgcagcgcggttaattcgttctggcgttgctgccagctctgcgcttcttgctgacgtgtcgccaaccagctctcttcttcatcttcctgtggcaatgtcagtgcataacccgtcaatgtcgttaaaagtagttgctggcgttgttcaatttgctgttgatactggataatttgctgattatgcgcggcaatctgcccttgtaattcatgccgttggctgagtaaccgcagctggcgttcgtgctcatcttgtgcatccagccacggttgaatatcgtccagtggctgcaaggtgatattgaggctggccgtgacggcttgccattgttgagtaagtgcttgctcatcttgtcggaggctttgcgcttcgttttcatcacgctgaagctgctttgttatggcgtccagttgcccacgtagcgtcgcaccttcttcaccgagctttttaacttcgttttccagcgccagtaatcgagactgattaacgccaggctccagcgcctgatacgcctcgaccgccgggtggctggtggaaccacaaagtgggcaaggctgacccgcctgtaactgtgcacgttgagcttccagcgttttgatgcgcgcttcctgctcgcaaatggttttcacatcggcaagttgctgcgtcttttctttataacgctggcgcatttcgttaagtgcggcgttacgttgcgtctgttcttgcgtgacattctggatagcgacctgtaactgcgccagacgtttttgttggggaacaatctgtccatgcagcgcgaccaggtgctgacgcagtgggcgttgctcagcatgttgcgccagggcggtagcaacttcatcggcggttaacgtcaacgtgatcgccgcaagcgcattaagtttttgctcagcatgggttaactgttgctgccattgccgcagatgctcgcgatcgctggtttgttgggagaactgcgcacgccaacccgccggttcgttgttccactgacggaagcggtcgtgttcctgtaaccaggtattcaggctttgttgctgctgctgtaattctgctgactgcttcgccgcgtggtggcgaatgctcgcgcgaagcgccattgtgctctgtaagcgagtatttacttcttcaatctgctggcgaatatgcgccagcgccgcgctgtgttctgcgatgcgttcccagtgtggacgaagatttcgtgccggttgtgccagactaagcgccgccagttgaggttgcgctttttcttcttcggctaacgcctgttgcaaggcctgctgacggcggctggcttcttgctgcaattcgtcctgacgcgttaaccagtttagcgattgttgttcttgctgctgcgcggtaattaactgtttttcttcgtcagtaagtacctgcaaactcgctgtcagcgattgcacttgttccggcgtgagcaacgtgacgccgctggcctgcgcttgcagcttctccagctctgtgcgggccgatttgtgctgctcaaaaaccatcgccgagatttgcccgtagatttcagtgccggttaactcctcgagcaattccgcgcgttctttgggtttggcattcaggaaggcagcaaattgcccctgcgaaagcagcatcgaacgggtgaagcgcccgtaatccagcccggttaacgtcgctgtcagttccagcttatctttcactttgtcggcgagaattttgccgtcggcgcagcgcgccagctctacgcgtggcacctgcaaattaccgtcgggttggttacgcgcccgattctggctccagaatgcacggtacgcttcacctttcacttcaaactccacctccgccagacattcggcggtatcgcgggtcatgagatcattttgcgattgtgaaacgttagagagacgcggagtttcgtgatacagcgccagacaaatggcgtccagcagggtggttttccccgcacctgttgggccggtaatagcaaacagcccgttgctggcgaacggctcgcgggtgaaatcaatcttccattcgccttttaatgagttcaggtttttcaggcgcaggctgagaattttcat

SEQ ID NO: 2 - DNA, 1203 bp, Escherichia coli
  source 1..1203: mol_type = other DNA
tcatgcttcgtgttctccggcgagggtatgcaacgtcgtggtgaaaagatgctgcagacgttgctgctgcgattcatccagttcttccagtgccagacggcgattgaacacctcttcgacgctgagttcgctgagggtttcacgctgttggctggctaacacacgctcgcgctgttcacgactccgacgtaccagcaatacttcgacaggcaatgattcggttaatgcctggattttgcgctgaatatcatgcagatactcatcagtagtgatttcgatatccagccagacaggtggctcctgcgatacatcgcgccactgttccagctgtgcggtaatcgacgccagatcgcctttcagcactgccatgggttgcgttaccggtacgttcaggttttccacgctctctaatttgccgtttgaaaatgtcaccagatggacatatttactcttaccgcattcatcaaaactcagtggaatgggggagccgcaatagcgaacatgttccatgccgccaataatctgtgcgcggtgaatatgcccgagcgcgatgtagtcggctggtggaaagttttgtgccggaaacgcgtccagcgtgccaatataaatgtcacgcacggcgtcacttttactggcccccacggtcgttaaatgtcccgtggcgatgatgggcagaggctgatcgccgcgcagtttgcaggcatcggcatagtgttgttggtaataatcggtaatcgctgccagtaaatgctgctgtttttcaataccgttaagccccgcctggctggtaataatgtcacgcggacgtaaaaacggaatggggcacagcactgcgcctggcgtcccgtcgcgacgaggcaagatttgcggcgcatgtccggcgctggcgaccacggtagtattgaggaacgccatgatatcgcgcgattcattcagcgtggcgaccgagtcatggtttcctgccagtaccaccagatgacagccagtttgctgtaaattgacaacaaaacggttgtataacgtgcgggcgtaactgggcggcgagccggtatcgaaaacatcaccggcaacaataatcgcatccacctgatgggtttgtgctgtctccagcagccagtcaagaaaagcctgatgttcagcttcgcggcttttactgtagaagttctggccgagatgccagtctgaggtgtgaaggatgcgcat

SEQ ID NO: 3 - DNA, 672 bp, Escherichia coli
  source 1..672: mol_type = other DNA
atggatctcgcgtcattacgcgctcaacaaatcgaactggcttcttctgtgatccgcgaggatcgactcgataaagatccaccggatctgatcgccggagccgatgtcgggtttgagcagggcggagaagtgacgcgagcggcgatggtgctgctgaaatatccctcgcttgagctggtcgagtataaagttgcccgcatcgccaccaccatgccttacattccaggttttctttccttccgcgaatatcctgcgctgctggcagcgtgggagatgctgtcgcaaaagccggatttagtgtttgtcgatggtcatgggatctcgcatcctcgccgtcttggcgtcgccagccattttggcttattggtggatgtgccgaccattggcgtggcgaaaaaacggctctgcggtaaattcgaaccgctctccagcgaaccgggcgcgctggccccactgatggataaaggcgagcagctggcctgggtctggcgcagcaaagcgcgctgtaacccgttgtttatcgctaccggccatcgggtcagcgtggacagcgcgctggcgtgggtacaacgctgcatgaaaggctatcgtctgccggagccaacgcgctgggcggacgcggtggcctcggaacgtccggcgttcgtgcgctatacagcaaatcagccctaa

SEQ ID NO: 4 - DNA, 1848 bp, Escherichia coli
  source 1..1848: mol_type = other DNA
atgccaattcaggtcttaccgccacaactggcgaaccagattgccgcaggtgaggtggtcgagcgacctgcgtcggtagtcaaagaactagtggaaaacagcctcgatgcaggtgcgacgcgtatcgatattgatatcgaacgcggtggggcgaaacttatccgcattcgtgataacggctgcggtatcaaaaaagatgagctggcgctggcgctggctcgtcatgccaccagtaaaatcgcctctctggacgatctcgaagccattatcagcctgggctttcgcggtgaggcgctggcgagtatcagttcggtttcccgcctgacgctcacttcacgcaccgcagaacagcaggaagcctggcaggcctatgccgaagggcgcgatatgaacgtgacggtaaaaccggcggcgcatcctgtggggacgacgctggaggtgctggatctgttctacaacaccccggcgcggcgcaaattcctgcgcaccgagaaaaccgaatttaaccacattgatgagatcatccgccgcattgcgctggcgcgtttcgacgtcacgatcaacctgtcgcataacggtaaaattgtgcgtcagtaccgcgcagtgccggaaggcgggcaaaaagaacggcgcttaggcgcgatttgcggcaccgcttttcttgaacaagcgctggcgattgaatggcaacacggcgatctcacgctacgcggctgggtggccgatccaaatcacaccacgcccgcactggcagaaattcagtattgctacgtgaacggtcgcatgatgcgcgatcgcctgatcaatcacgcgatccgccaggcctgcgaagacaaactgggggccgatcagcaaccggcatttgtgttgtatctggagatcgacccacatcaggtggacgtcaacgtgcaccccgccaaacacgaagtgcgtttccatcagtcgcgtctggtgcatgattttatctatcagggcgtgctgagcgtgctacaacagcaactggaaacgccgctaccgctggacgatgaaccccaacctgcaccgcgttccattccggaaaaccgcgtggcggcggggcgcaatcactttgcagaaccggcagctcgtgagccggtagctccgcgctacactcctgcgccagcatcaggcagtcgtccggctgccccctggccgaatgcgcagccaggctaccagaaacagcaaggtgaagtgtatcgccagcttttgcaaacgcccgcgccgatgcaaaaattaaaagcgccggaaccgcaggaacctgcacttgcggcgaacagtcagagttttggtcgggtactgactatcgtccattccgactgtgcgttgctggagcgcgacggcaacatttcacttttatccttgccagtggcagaacgttggctgcgtcaggcacaattgacgccgggtgaagcgcccgtttgcgcccagccgctgctgattccgttgcggctaaaagtttctgccgaagaaaaatcggcattagaaaaagcgcagtctgccctggcggaattgggtattgatttccagtcagatgcacagcatgtgaccatcagggcagtgcctttacccttacgccaacaaaatttacaaatcttgattcctgaactgataggctacctggcgaagcagtccgtattcgaacctggcaatattgcgcagtggattgcacgaaatctgatgagcgaacatgcgcagtggtcaatggcacaggccataaccctgctggcggacgtggaacggttatgtccgcaacttgtgaaaacgccgccgggtggtctgttacaatctgttgatttacatccggcgataaaagccctgaaagatgagtga

SEQ ID NO: 5 - DNA, 612 bp, Escherichia coli
  source 1..612: mol_type = other DNA
tcataacgcggcgcgtagggcttcgcgaattaaagtttcactgctggcgtcagggcgagcgattttgctcaccatgcggcttgcttcttgtggtttatagcccagcgccaccagcgcggcaaccgcttcttgttcagcatcgtcggtcgccgggctggcaggagacgtgagtaccaggtcggcggctggcgtaaagagatcgccatgcaaacctttaaatcggtctttcatttcaacaatcaagcgttcggcggtttttttgccaatacccggcagtttcaccagtgcccccacttcttcacgctcaacggcattaacgaactgctgcgctgacattccggagaggatcgccagcgccaacttcgggccgacgccgttggttttgatcaactctttgaacaatgtgcgctcttgtttattgttaaaaccgtacagcagttgcgcgtcttcacgcaccacaaagtgggtgaaaacgatcgcttcctgacccgcttcagggagttcataaaaacaggtcatcggcatatgcacttcatagcctacgccgcccacttcaattaacaccagcgggggttgtttttcaatgatgatgcctctgagtctgcctatcac

SEQ ID NO: 6 - DNA, 1011 bp, Escherichia coli
  source 1..1011: mol_type = other DNA
ttacggcatttctggcggcgttatgccaaagtgattccacgcccgcgtcgtcgccatacgcccacgcggtgtacgctgcaaaaagccttgctgaatcaaataaggttccagcacatcctcaatggtttcacgttcttcgccaatggctgccgccaggttatccagacctacaggtccaccaaagaacttatcgattaccgccagcaacaatttgcggtccatataatcgaaaccttcagcatcgacattcaacatatccagcgcctgagcagcgatatctgccgagatggtgccatcgtgcttcacttcggcgaaatcacgcactcgacgcagcagacggttggcaatgcgcggcgtaccgcgagcgcgacgagcaacttccagcgcgccgtcatcactcatctcaagccccataaagcgtgcgctgcgactgacgatatattgcagatccggcacctgataaaactccagacgttgcacaataccaaaacggtcgcgcaacggtgatgtcagcgaacctgcgcgcgtggttgcaccaatcagggtaaacggcggcaaatcaattttaatggagcgtgccgccggaccttcaccaatcatgatatccagttggtagtcttccattgccgggtacagcacttcttcaacaactggcgatagacggtggatctcatcaataaacagcacgtcatgcggttcaaggttagtgagcatcgcagccaaatcgcccgccttttccagcaccggaccagaagtcgtgcgtaaattaacgcccatttcattggcgacaatgttggcaagcgtagttttacccaaccccggaggaccaaaaatcaacaaatgatcgagggcatcgccgcgcagtttcgctgctttgatgaaaatctccatctgtgaacgaacctgcggctgaccaacatactcttccagtaatttggggcgaatggcgcgatctgctacatcttccggcaaagtggtaccggcagaaatcagacggtctgcttcaatcat

SEQ ID NO: 7 - DNA, 522 bp, Escherichia coli
  source 1..522: mol_type = other DNA
ttaacgcagtcgccctctcgccaggttcagccgcgattcgctcatctgcatcgcattctgactaacgtggcagtgggtgatagcaatcgccagcgcatcggcggcatccgcctgtggattagcgggcagtttcagcaaggtgcggaccatatgctgcacctggcttttttcggcactgccaatacctaccaccgtttgctttacctgacgtgccgcgtattcaaatactggcaactcctgattcaccgccgccacaatcgccacgccgcgcgcctggcccagtttcagggctgagtcagcgttctttgccataaagacttgttcaatggcgaaataatcaggctggaactgggtgatgatttccgtcacgcccgcatagatgagtttcagacgagacggtaaatcatccactttggtgcggatgcatccgctacccaggtaggacagttgcctacctacctggcggatgacgccgtagccggtcacgcgcgaacccggatcaatgccgagaataatagccat

SEQ ID NO: 8 - DNA, 1083 bp, Escherichia coli
  source 1..1083: mol_type = other DNA
tcactgcccgctttccagtcgggaaacctgtcgtgccagctgcattaatgaatcggccaacgcgcggggagaggcggtttgcgtattgggcgccagggtggtttttcttttcaccagtgagacgggcaacagctgattgcccttcaccgcctggccctgagagagttgcagcaagcggtccacgctggtttgccccagcaggcgaaaatcctgtttgatggtggttaacggcgggatataacatgagctgtcttcggtatcgtcgtatcccactaccgagatatccgcaccaacgcgcagcccggactcggtaatggcgcgcattgcgcccagcgccatctgatcgttggcaaccagcatcgcagtgggaacgatgccctcattcagcatttgcatggtttgttgaaaaccggacatggcactccagtcgccttcccgttccgctatcggctgaatttgattgcgagtgagatatttatgccagccagccagacgcagacgcgccgagacagaacttaatgggcccgctaacagcgcgatttgctggtgacccaatgcgaccagatgctccacgcccagtcgcgtaccgtcttcatgggagaaaataatactgttgatgggtgtctggtcagagacatcaagaaataacgccggaacattagtgcaggcagcttccacagcaatggcatcctggtcatccagcggatagttaatgatcagcccactgacgcgttgcgcgagaagattgtgcaccgccgctttacaggcttcgacgccgcttcgttctaccatcgacaccaccacgctggcacccagttgatcggcgcgagatttaatcgccgcgacaatttgcgacggcgcgtgcagggccagactggaggtggcaacgccaatcagcaacgactgtttgcccgccagttgttgtgccacgcggttgggaatgtaattcagctccgccatcgccgcttccactttttcccgcgttttcgcagaaacgtggctggcctggttcaccacgcgggaaacggtctgataagagacaccggcatactctgcgacatcgtataacgttactggtttcac

SEQ ID NO: 9 - DNA, 1139 bp, Escherichia coli
  source 1..1139: mol_type = other DNA
acctttcgcggtatggcatgatagcgcccggaagagagtcaattcagggtggtgaatgtgaaaccagtaacgttatacgatgtcgcagagtatgccggtgtctcttatcagaccgtttcccgcgtggtgaaccaggccagccacgtttctgcgaaaacgcgggaaaaagtggaagcggcgatggcggagctgaattacattcccaaccgcgtggcacaacaactggcgggcaaacagtcgttgctgattggcgttgccacctccagtctggccctgcacgcgccgtcgcaaattgtcgcggcgattaaatctcgcgccgatcaactgggtgccagcgtggtggtgtcgatggtagaacgaagcggcgtcgaagcctgtaaagcggcggtgcacaatcttctcgcgcaacgcgtcagtgggctgatcattaactatccgctggatgaccaggatgccattgctgtggaagctgcctgcactaatgttccggcgttatttcttgatgtctctgaccagacacccatcaacagtattattttctcccatgaagacggtacgcgactgggcgtggagcatctggtcgcattgggtcaccagcaaatcgcgctgttagcgggcccattaagttctgtctcggcgcgtctgcgtctggctggctggcataaatatctcactcgcaatcaaattcagccgatagcggaacgggaaggcgactggagtgccatgtccggttttcaacaaaccatgcaaatgctgaatgagggcatcgttcccactgcgatgctggttgccaacgatcagatggcgctgggcgcaatgcgcgccattaccgagtccgggctgcgcgttggtgcgatatctcggtagtgggatacgacgataccgaagacagctcatgttatatcccgccgttaaccaccatcaaacaggattttcgcctgctggggcaaaccagcgtggaccgcttgctgcaactctctcagggccaggcggtgaagggcaatcagctgttgcccgtctcactggtgaaaagaaaaaccacgctagcgcccaatacgcaaaccgcctctccccgcgcgttggccgattcattaatgcagctggcacgacaggtttcccgactggaaagcgggcagtga

SEQ ID NO: 10 - DNA, 145 bp, Adeno-associated virus
  source 1..145: mol_type = other DNA
aggaacccctagtgatggagttggccactccctctctgcgcgctcgctcgctcactgaggccgcccgggcaaagcccgggcgtcgggcgacctttggtcgcccggcctcagtgagcgagcgagcgcgcagagagggagtggccaa

SEQ ID NO: 11 - DNA, 20 bp, synthetic construct
  source 1..20: mol_type = other DNA
ttccgcgcgttctttgggtt

SEQ ID NO: 12 - DNA, 20 bp, synthetic construct
  source 1..20: mol_type = other DNA
cgattgaacacctcttcgac

SEQ ID NO: 13 - DNA, 20 bp, synthetic construct
  source 1..20: mol_type = other DNA
atctcgcatcctcgccgtct

SEQ ID NO: 14 - DNA, 20 bp, synthetic construct
  source 1..20: mol_type = other DNA
attatcagcctgggctttcg

SEQ ID NO: 15 - DNA, 20 bp, synthetic construct
  source 1..20: mol_type = other DNA
ttcaacaatcaagcgttcgg

SEQ ID NO: 16 - DNA, 20 bp, synthetic construct
  source 1..20: mol_type = other DNA
cggaggaccaaaaatcaaca

SEQ ID NO: 17 - DNA, 20 bp, synthetic construct
  source 1..20: mol_type = other DNA
tgcggaccatatgctgcacc

SEQ ID NO: 18 - DNA, 20 bp, synthetic construct
  source 1..20: mol_type = other DNA
gatgaacgtgccggaaagcg

SEQ ID NO: 19 - DNA, 20 bp, synthetic construct
  source 1..20: mol_type = other DNA
gccggataagcctcgctttc

SEQ ID NO: 20 - DNA, 125 bp, synthetic construct
  source 1..125: mol_type = other DNA
ttggccactccctctctgcgcgctcgctcgctcactgaggccgggcgaccaaaggtcgcccgacgcccgggctttgcccgggcggcctcagtgagcgagcgagcgcgcagagagggagtggccaa

SEQ ID NO: 21 - DNA, 119 bp, synthetic construct
  source 1..119: mol_type = other DNA
gccactccctctctgcgcgctcgctcgctcactgaggccgggcgaccaaaggtcgcccgacgcccgggctttgcccgggcggcctcagtgagcgagcgagcgcgcagagagggagtggc

SEQ ID NO: 22 - DNA, 1003 bp, synthetic construct
  source 1..1003: mol_type = other DNA
cacgatcgctccgacgccaaaaaatgcgccatgcggaaagccggataccagccgaccaatggcgagcatcaggtaagacgaagagagcgtgaacatggcgttgccaatgacgcacaacgccaccagaaacaacaagatatgtttgagtgagtagcggctggaaaagagtgcgatgattggcgcaccgaccaccacccccagtgcataatacgagatcatatgcccggcggcaggaatcgaaattcctacgttatgcgccagctccgtgagcacgcccataatgccaaattcggccatccccaaaccaaacgtgcccagagccaaagataaaatgacttttttcataccaccatcacaaccaccagaacggctaccaatcaccgtagccaataaagtgatagcttgcaggataacgaccagcaaggccaagagataattcgcccctctgtattcattatcctgctgaatagttatttcactgcaaacgtactttccagtttgctcccgttgctggcgaacggctcgcgggtgaaatcaatcttccattcgccttttaatgagttcaggtttttcaggcgcaggctgagaattttcatgcttcgtgttctccggcgagggtatgcaacgtcgtggtgaaaagatgctgcagacgttgctgctgcgattcatccagttcttccagtgccagacggcgattgaacacctcttcgacgctgagttcgctgagggtttcacgctgttggctggctaacacacgctcgcgctgttcacgactccgacgtaccagcaatacttcgacaggcaatgattcggttaatgcctggattttgcgctgaatatcatgcagatactcatcagtagtgatttcgatatccagccagacaggtggctcctgcgatacatcgcgccactgttccagctgtgcggtaatcgacgccagatcgcctttcagcactgccatgggttgcgttaccggtacgttcaggttttccacgctctctaa

SEQ ID NO: 23 - DNA, 1000 bp, synthetic construct
  source 1..1000: mol_type = other DNA
cgtcgctgtcagttccagcttatctttcactttgtcggcgagaattttgccgtcggcgcagcgcgccagctctacgcgtggcacctgcaaattaccgtcgggttggttacgcgcccgattctggctccagaatgcacggtacgcttcacctttcacttcaaactccacctccgccagacattcggcggtatcgcgggtcatgagatcattttgcgattgtgaaacgttagagagacgcggagtttcgtgatacagcgccagacaaatggcgtccagcagggtggttttccccgcacctgttgggccggtaatagcaaacagcccgttgctggcgaacggctcgcgggtgaaatcaatcttccattcgccttttaatgagttcaggtttttcaggcgcaggctgagaattttcatgcttcgtgttctccggcgagggtatgcaacgtcgtggtgaaaagatgctgcagacgttgctgctgcgattcatccagttcttccagctggccgagatgccagtctgaggtgtgaaggatgcgcataacggttccctggcgaaaaagcatgggcgcgattatacccaaacagatgtgccatttgcttttttctgcgccacggaaatcaataacctgaagatatgtgcgacgagcttttcataaatctgtcataaatctgacgcataatgacgtcgcattaatgatcgcaacctatttattacaacagggcaaatcatggcgagacgtattctggtcgtagaagatgaagctccaattcgcgaaatggtctgcttcgtgctcgaacaaaatggctttcagccggtcgaagcggaagattatgacagtgctgtgaatcaactgaatgaaccctggccggatttaattctcctcgactggatgttacctggcggctccggtatccagttcatcaaacacctcaagcgcgagtcgatgacccgggatattccagtggtgatgttgaccgccagaggggaagaagaagatcg

SEQ ID NO: 24 - DNA, 1000 bp, synthetic construct
  source 1..1000: mol_type = other DNA
aacagttctcgctctattacatgcataaaattgttgatggtttactgcgtgaaaacgacggtcgccgcgtaccggtcacgctgtttaccaaaggcggcggacagtggctggaagccatggcagaaaccggttgcgatgcgctgggcctcgactggacaacggacatcgccgatgcgcgccgccgtgtgggcaataaagtcgcgttgcagggtaatatggatccgtcgatgctgtacgcgccgcctgcccgcattgaagaagaagtagcgactatacttgcaggtttcggtcacggcgaaggtcatgtctttaaccttggtcacggcattcatcaggatgtgccgccagaacatgctggcgtgttcgtggaggcagtgcatcgactgtctgaacagtatcaccgctaaggagtgattatggatctcgcgtcattacgcgctcaacaaatcgaactggcttcttctgtgatccgcgaggatcgactcgataaagatccaccgcgtctgccggagccaacgcgctgggcggacgcggtggcctcggaacgtccggcgttcgtgcgctatacagcaaatcagccctaattcaggtaaactgcggataatttccgtatttgagaactcaacatgttacaaaacccaattcatctgcgtctggagcgcctggaaagctggcagcatgtcactttcatggcttgcttatgcgaacgcatgtaccccaattacgccatgttctgccagcaaaccggttttggtgatgggcaaatttaccgtcgcattctcgatctcatctgggaaacgctgaccgttaaagacgcaaaagtaaatttcgacagccaactggagaaatttgaagaagcgattccttcagccgacgatttcgatctgtacggcgtttatccggcaatcgatgcctgcgtggcgttaagtgaactggtccattcgcgtttgagtggtgaaacgctcgaacacgcggtggaagtgagtaagacctccatcac

SEQ ID NO: 25 - DNA, 1000 bp, synthetic construct
  source 1..1000: mol_type = other DNA
tgctgggtggggcgggtgatgtgctggcgaacagtcagtctgacccctatttaagccaggcggtgctggatttacagttcggtcattcccagcgggtagggtatgatgtagcgaccagtatgatcagtcagttgcaacgcattggcgaaatacataaacgtcgaccagaacacgccagccttggcgttctgcgctcgccggatatcccatcagtactggtcgaaaccggttttatcagcaacaacagcgaagaacgtttgctggcgagcgacgattaccaacaacagctggcagaagccatttacaaaggcctgcgcaattacttccttgcgcatccgatgcaatctgcgccgcagggtgcaacggcacaaactgccagtacggtgacgacgccagatcgcacgctgccaaactaaggacgattgatgccaattcaggtcttaccgccacaactggcgaaccagattgccgcaggtgaggtggtcgagcgacctgcgtcgcttgtgaaaacgccgccgggtggtctgttacaatctgttgatttacatccggcgataaaagccctgaaagatgagtgatatcagtaaggcgagcctgcctaaggcgatttttttgatggggccgacggcctccggtaaaacggcgttagccattgagctgcgtaaaattttaccagtagagttgataagcgttgattctgcccttatttacaaagggatggatatcgggacggcgaagccgaacgctgaagagttactcgccgcgccgcaccgattgctggatattcgcgatccgtcgcaggcttactcggctgctgattttcgccgcgatgcgctggcggaaatggccgatatcaccgcggcggggcggatcccactgttagtgggcggtacgatgttgtatttcaaggcattgctggaagggttgtcgccgctaccgtcggcagacccggaagtacgggccagaattgagcaacaggcggcagagcaaggttgggagt

SEQ ID NO: 26 - DNA, 1000 bp, synthetic construct
  source 1..1000: mol_type = other DNA
cggcaaatcaattttaatggagcgtgccgccggaccttcaccaatcatgatatccagttggtagtcttccattgccgggtacagcacttcttcaacaactggcgatagacggtggatctcatcaataaacagcacgtcatgcggttcaaggttagtgagcatcgcagccaaatcgcccgccttttccagcaccggaccagaagtcgtgcgtaaattaacgcccatttcattggcgacaatgttggcaagcgtagttttacccaaccccggaggaccaaaaatcaacaaatgatcgagggcatcgccgcgcagtttcgctgctttgatgaaaatctccatctgtgaacgaacctgcggctgaccaacatactcttccagtaatttggggcgaatggcgcgatctgctacatcttccggcaaagtggtaccggcagaaatcagacggtctgcttcaatcatcctttacctcataacgcggcgcgtagggcttcgcgaattaacatatgcacttcatagcctacgccgcccacttcaattaacaccagcgggggttgtttttcaatgatgatgcctctgagtctgcctatcacatgacgctcctgcgtaatgaatcaaagataatgctgtatgataaaaaaatgctggatagatatccagcgaaggatgaagaaaacttgcgaggtgtctcgatgaactgaaaaatggcacagtataatttattctacaggttatattggaagcaaatattttaatattacatattcagtgaagaaatgcgtaataaaaatatacattgcgcctcctgaaaaaataaattttttatgctattacgtatatttgtatctatttcaatggaatgacaacgtgaatattaattaccctgctgaatatgaaattggagatatcgtctttacatgtataggtgctgccttatttggtcaaatatcagctgcatcaaattgctggagtaatcacgtcgggatcattatcggtcataacg

SEQ ID NO: 27 - DNA, 1000 bp, synthetic construct
  source 1..1000: mol_type = other DNA
cgagtgaaattgttgttgatgctggtgacggcattgacgattggtgtagcgatgaaatttgtcggtgcgttgattattacttcgttgctgattattcctgctgctactgcgcgtcgctttgcccgcacgccggaacagatggctggtgtcgctgttttggtggggatggtggcagtgactggcggtttaaccttttccgcggtttacgatacgccggcgggtccgtcggtggtgctatgtgcggcactgttatttattctcagtatgatgaaaaagcaggccagctaatctatcgctgaacacatttgtcggatgcggcgcgagcgccttatccgacctacggttcggtatctctggtagtcctggtaagacgcgaacagcgtcgcatcaggcatattgccagtgccggatgcggcgcgagcgaccaatccgacttacggcatttctggcggcgttatgccaaagtgattccacgcccgcgtcgtcgccatacgcccacggcgaatggcgcgatctgctacatcttccggcaaagtggtaccggcagaaatcagacggtctgcttcaatcatcctttacctcataacgcggcgcgtagggcttcgcgaattaaagtttcactgctggcgtcagggcgagcgattttgctcaccatgcggcttgcttcttgtggtttatagcccagcgccaccagcgcggcaaccgcttcttgttcagcatcgtcggtcgccgggctggcaggagacgtgagtaccaggtcggcggctggcgtaaagagatcgccatgcaaacctttaaatcggtctttcatttcaacaatcaagcgttcggcggtttttttgccaatacccggcagtttcaccagtgcccccacttcttcacgctcaacggcattaacgaactgctgcgctgacattccggagaggatcgccagcgccaacttcgggccgacgccgttggttttgatcaactctttgaacaatgtgcgctcttgtttatt

SEQ ID NO: 28 - DNA, 1000 bp, synthetic construct
  source 1..1000: mol_type = other DNA
aagccgggttcccctttcaaccatcaccacgctatctcgttttattaaacgttcgtctaatcaacgctatgctataaagcgattagacgctgggctgacagaacgacaaaaacaacgaattgttgaacaggttccctcccggctacgcaaactttaccacaccggttttaaatacgaatcttcgcgccagttctgttcaaaatttgtttttgatatttataaagaagcgctatgtattccggtgggtgaaatagagacgtttggagaattgttaaatagcaatccgaatgcaaaactcactttctggaaattctggttcctgggttctattccgtgggagcgtaaaaccgtcacgccagccagtttgtggcatcatccgggtttggtgttgattcatgcggagggagtggaaacgcctcagccggaactgaccgaggcggtataacttaacgcagtcgccctctcgccaggttcagccgcgattcgctcatctgcatcgcggtcacgcgcgaacccggatcaatgccgagaataatagccatcacgcgtctccgttttgctgtttagcaggcctcatcagagagtcgctgcgacctcatcagagatttcaccgttatggtaaacttcctgcacgtcgtcgcaatcttccagcatatcgatcagacgcatcagtttcggtgcggtttctgcatccatatcagctttggtagacgggatcatggaaacttccgcgctgtctgctttcagacctgccgcttccagagcgtcgcgcactttacccatttcttcccatgcagtgtagacatcaatcgcgccgtcatcataggtcacaacgtcttcagcacctgcttccagtgctgcttccatgatggtgtcttcatcgcctttctcgaaggagatcacgccttttttgctgaacagataggcaacggaaccatcagtaccgaggttaccgccacatttgctaaatgcatgacgcacttcagcaacggtacggttg

SEQ ID NO: 29 - DNA, 2417 bp, synthetic construct
  source 1..2417: mol_type = other DNA
tggttatcgatatcatgatactgcggcggggcgctaaaacgaagggaagaagcattagtgtaattaattaaagcaagataatacgtatgtttgatcaattttcgaggcgataaccggccataaaaaagcgcaacgtagaacaggaattattctcacgaaagaaatccattaccatctctttatccagtccatagcggcgcgtcagaatacccgcttcccaggcgctaagctggcgatctccggtcttttcgtacatccggtgtgagtagcctaatacaaaaccgcgtttataatcggcacagaattttgtcacattaaccgcactgtcggcatgcgttgcttttaatcccgccattaagcctttaccaaaatggttattcatcgttcacctcattcgctatatattgtcatatatagcgatattttaggcaaagaacgacttttgcgcacgctattttttcatgcttgtttaagacgtaatcccgtaagagataaacctattccgacaccatcgaatggtgcaaaacctttcgcggtatggcatgatagcgcccggaagagagtcaattcagggtggtgaatgtgaaaccagtaacgttatacgatgtcgcagagtatgccggtgtctcttatcagaccgtttcccgcgtggtgaaccaggccagccacgtttctgcgaaaacgcgggaaaaagtggaagcggcgatggcggagctgaattacattcccaaccgcgtggcacaacaactggcgggcaaacagtcgttgctgattggcgttgccacctccagtctggccctgcacgcgccgtcgcaaattgtcgcggcgattaaatctcgcgccgatcaactgggtgccagcgtggtggtgtcgatggtagaacgaagcggcgtcgaagcctgtaaagcggcggtgcacaatcttctcgcgcaacgcgtcagtgggctgatcattaactatccgctggatgaccaggatgccattgctgtggaagctgcctgcactaatgttccggcgttatttcttgatgtctctgaccagacacccatcaacagtattattttctcccatgaagacggtacgcgactgggcgtggagcatctggtcgcattgggtcaccagcaaatcgcgctgttagcgggcccattaagttctgtctcggcgcgtctgcgtctggctggctggcataaatatctcactcgcaatcaaattcagccgatagcggaacgggaaggcgactggagtgccatgtccggttttcaacaaaccatgcaaatgctgaatgagggcatcgttcccactgcgatgctggttgccaacgatcagatggcgctgggcgcaatgcgcgccattaccgagtccgggctgcgcgttggtgcggatatctcggtagtgggatacgacgataccgaagacagctcatgttatatcccgccgttaaccaccatcaaacaggattttcgcctgctggggcaaaccagcgtggaccgcttgctgcaactctctcagggccaggcggtgaagggcaatcagctgttgcccgtctcactggtgaaaagaaaaaccaccctggcgcccaatacgcaaaccgcctctccccgcgcgttggccgattcattaatgcagctggcacgacaggtttcccgactggaaagcgggcagtgaaattcgcgcaacgcaattaatgtaagttagctcactcattaggcaccaaataaaacgaaaggctcagtcgaaagactgggcctttcgttttatctgttgtttgtcggtgaacgctctcctgagtaggacaaatccgccgggagcggatttgaacgttgcgaagcaacggcccggagggtggcgggcaggacgcccgccataaactgccaggcatcaaattaagcagaaggccatcctgacggatggccttttagtaatccagcaactcttgtgggaaatctttggcggttaaacgcggcatcgttgcactcctcagttggtgtttttttaagcaaagcataagcacgtatttttgcccagtttttcgtcactctgtgagccagactacgggatacgcgctggcgaatcgctaaactagaaacattgtttcgaaattgaacggtggaaaggagaggtcatggtctggttagcgaatcccgaacgttacgggcagatgcaataccgctattgcggaaaaagtggtttacgcctgcccgcgttatcgctcggtttatggcacaatttcggtcacgttaacgcgctggaatcacagcgtgcgatcctgcgtaaagcgtttgatttgggcattacgcactttgatttagccaacaattacgggccgcctccaggaagcgcagaagagaactttggtcgcctgctgcgggaggattttgccgcttatcgcgatgaactgattatctctaccaaggctg

SEQ ID NO: 30 - DNA, 2410 bp, synthetic construct
  source 1..2410: mol_type = other DNA
caaacctgggggttgttcttcgaacgcctgaatgtatcggtacagaaactggaaaacgccatcgagttttatggcgcgatttcgcataacaaactgcacggcctgtcagtgcaggttgaaaccaatcacgtcaaattaccggcggtggtggacggctttgccagcgaagggatcatccagttctttttcgaagaaacgcaagacgagaatggctttaatatctacattctcgacgaaagcaaccgggttgaggtatatcaccactgcgaaggcagcaaagaggagctggtacgtgacgtcagtcgcttctactcgtcatcgcatgaccgctttacctacggctcaagcttcatcaacttcaacctgccgcagttctatcagattgtgaaggttgatggtcgtgaacaggtgattccgttccgcacaaaatctatcggtaacatgccgcctgccaatcaggatcacgatacgccgctattacagcaatatttttcgtgatgaacgtggacaccatcgaatggtgcaaaacctttcgcggtatggcatgatagcgcccggaagagagtcaattcagggtggtgaatgtgaaaccagtaacgttatacgatgtcgcagagtatgccggtgtctcttatcagaccgtttcccgcgtggtgaaccaggccagccacgtttctgcgaaaacgcgggaaaaagtggaagcggcgatggcggagctgaattacattcccaaccgcgtggcacaacaactggcgggcaaacagtcgttgctgattggcgttgccacctccagtctggccctgcacgcgccgtcgcaaattgtcgcggcgattaaatctcgcgccgatcaactgggtgccagcgtggtggtgtcgatggtagaacgaagcggcgtcgaagcctgtaaagcggcggtgcacaatcttctcgcgcaacgcgtcagtgggctgatcattaactatccgctggatgaccaggatgccattgctgtggaagctgcctgcactaatgttccggcgttatttcttgatgtctctgaccagacacccatcaacagtattattttctcccatgaagacggtacgcgactgggcgtggagcatctggtcgcattgggtcaccagcaaatcgcgctgttagcgggcccattaagttctgtctcggcgcgtctgcgtctggctggctggcataaatatctcactcgcaatcaaattcagccgatagcggaacgggaaggcgactggagtgccatgtccggttttcaacaaaccatgcaaatgctgaatgagggcatcgttcccactgcgatgctggttgccaacgatcagatggcgctgggcgcaatgcgcgccattaccgagtccgggctgcgcgttggtgcggatatctcggtagtgggatacgacgataccgaagacagctcatgttatatcccgccgttaaccaccatcaaacaggattttcgcctgctggggcaaaccagcgtggaccgcttgctgcaactctctcagggccaggcggtgaagggcaatcagctgttgcccgtctcactggtgaaaagaaaaaccacgctagcgcccaatacgcaaaccgcctctccccgcgcgttggccgattcattaatgcagctggcacgacaggtttcccgactggaaagcgggcagtgagcgcaacgcaattaatgtaagttagctcactcattaggcaccaaataaaacgaaaggctcagtcgaaagactgggcctttcgttttatctgttgtttgtcggtgaacgctctcctgagtaggacaaatccgccgggagcggatttgaacgttgcgaagcaacggcccggagggtggcgggcaggacgcccgccataaactgccaggcatcaaattaagcagaaggccatcctgacggatggccttttatgcaatcttagcggaaactgactgtttcacccgcctgctgcgtcgccgcctgttccagcaaatcccagaaggtttcgccgctgcgatcacaaatccactcatcgcctttcaggtcaaaatggtagccgccctgtttggttgccagccatacctggtgcagcggctcctggcggttgataatgattttgctgccattctcaaaggtaatggtcagtacgccgccgttgatttcgcagtcgatatcgctgtcgccatcccagtcgtccaggcgttcttcaatggtcagccagagttgatcagccaggcgatgaaattcactgtcgttcattgttgtatcctgtttttaagtgatggcggcagtatagcggcatggggtcagggcttcaaagtttgcacctctgcggctgcgttccggcacgattcatccgtcaccggaataatgatgtctctgtgtagcgaaagatttgtctcttcattagggcgcagttacaccac

SEQ ID NO: 31 - DNA, 27 bp, synthetic construct
  source 1..27: mol_type = other DNA
gcatgacaccggacattatcctgcagc

SEQ ID NO: 32 - DNA, 27 bp, synthetic construct
  source 1..27: mol_type = other DNA
tccccaaatacaaaaccaatttcagcc

SEQ ID NO: 33 - DNA, 30 bp, synthetic construct
  source 1..30: mol_type = other DNA
cggaatgcccagcaaattggcgactgtcat

SEQ ID NO: 34 - DNA, 30 bp, synthetic construct
  source 1..30: mol_type = other DNA
caccagctccttcggcgaaaacggcttggt

SEQ ID NO: 35 - DNA, 25 bp, synthetic construct
  source 1..25: mol_type = other DNA
caacagtgaaatggccagctggctg

SEQ ID NO: 36 - DNA, 32 bp, synthetic construct
  source 1..32: mol_type = other DNA
cgtcagttccgttaaagttttacccgaaatga

SEQ ID NO: 37 - DNA, 31 bp, synthetic construct
  source 1..31: mol_type = other DNA
tcactttgtatctgaatgcgcagattaaagc

SEQ ID NO: 38 - DNA, 32 bp, synthetic construct
  source 1..32: mol_type = other DNA
ttgctctacagctgggttttctttaagctctt

SEQ ID NO: 39 - DNA, 21 bp, synthetic construct
  source 1..21: mol_type = other DNA
gtttgttgatggtgtgaaatt

SEQ ID NO: 40 - DNA, 20 bp, synthetic construct
  source 1..20: mol_type = other DNA
caaccgcaaccgtaccgttg

SEQ ID NO: 41 - DNA, 25 bp, synthetic construct
  source 1..25: mol_type = other DNA
ccagcacccgccaggaaaccgggcg

SEQ ID NO: 42 - DNA, 24 bp, synthetic construct
  source 1..24: mol_type = other DNA
gctttatgcactatcgcaatgtgg

SEQ ID NO: 43 - DNA, 30 bp, synthetic construct
  source 1..30: mol_type = other DNA
ccagcacccgccaggaaaccgggcgtttca

SEQ ID NO: 44 - DNA, 30 bp, synthetic construct
  source 1..30: mol_type = other DNA
ggcgcgaggtgccgatcacgaaactaccag